European Patent Application EP 4 538 381 A1, published April 16, 2025. Title: 항원 단백질 또는 상기 단백질을 암호화하는 유전자를 포함하는 세포외소포체 및 그의 용도. Applicant: (주)엑솔런스. The sequence listing filed with the application follows.

SEQUENCE LISTING (3 sequences)

SEQ ID NO: 1 - protein, 566 aa, Influenza virus
MKAILVVLLYTFATANADTLCIGYHANNSTDTVDTVLEKNVTVTHSVNLLEDKHNGKLCKLRGVAPLHLGKCNIAGWILGNPECESLSTASSWSYIVETSSSDNGTCYPGDFIDYEELREQLSSVSSFERFEIFPKTSSWPNHDSNKGVTAACPHAGAKSFYKNLIWLVKKGNSYPKLSKSYINDKGKEVLVLWGIHHPSTSADQQSLYQTADAYVFVGTSRYSKKFKPEIAIRPKVRDQEGRMNYYWTLVEPGDKITFEATGNLVVPRYAFAMERNAGSGIIISDTPVHDCNTTCQTPKGAINTSLPFQNIHPITIGKCPKYVKSTKLRLATGLRNVPSIQSRGLFGAIAGFIEGGWTGMVDGWYGYHHQNEQGSGYAADLKSTQNAIDEITNKVNSVIEKMNTQFTAVGKEFNHLEKRIENLNKKVDDGFLDIWTYNAELLVLLENERTLDYHDSNVKNLYEKVRSQLKNNAKEIGNGCFEFYHKCDNTCMESVKNGTYDYPKYSEEAKLNREEIDGVKLESTRIYQILAIYSTVASSLVLVVSLGAISFWMCSNGSLQCRICI

SEQ ID NO: 2 - protein, 515 aa, Human respiratory syncytial virus
MQNITEEFYQSTCSAVSKGYLSALRTGWYTSVITIELSNIKENKCNGTDAKVKLIKQELDKYKNAVTELQLLMQSTPPTNNRARRELPRFMNYTLNNAKKTNVTLSKKRKRRFLGFLLGVGSAIASGVAVSKVLHLEGEVNKIKSALLSTNKAVVSLSNGVSVLTSKVLDLKNYIDKQLLPIVNKQSCSISNIETVIEFQQKNNRLLEITREFSVNAGVTTPVSTYMLTNSELLSLINDMPITNDQKKLMSNNVQIVRQQSYSIMSIIKEEVLAYVVQLPLYGVIDTPCWKLHTSPLCTTNTKEGSNICLTRTDRGWYCDNAGSVSFFPQAETCKVQSNRVFCDTMNSLTLPSEINLCNVDIFNPKYDCKIMTSKTDVSSSVITSLGAIVSCYGKTKCTASNKNRGIIKTFSNGCDYVSNKGMDTVSVGNTLYYVNKQEGKSLYVKGEPIINFYDPLVFPSDEFDASISQVNEKINQSLAFIRKSDELLHNVNAGKSTTNIMITTHHHHHHHHHH

SEQ ID NO: 3 - protein, 642 aa, Varicella-Zoster virus
MGTVNKPVVGVLMGFGIITGTLRITNPVRASVLRYDDFHIDEDKLDTNSVYEPYYHSDHAESSWVNRGESSRKAYDHNSPYIWPRNDYDGFLENAHEHHGVYNQGRGIDSGERLMQPTQMSAQEDLGDDTGIHVIPTLNGDDRHKIVNVDQRQYGDVFKGDLNPKPQGQRLIEVSVEENHPFTLRAPIQRIYGVRYTETWSFLPSLTCTGDAAPAIQHICLKHTTCFQDVVVDVDCAENTKEDQLAEISYRFQGKKEADQPWIVVNTSTLFDELELDPPEIEPGVLKVLRTEKQYLGVYIWNMRGSDGTSTYATFLVTWKGDEKTRNPTPAVTPQPRGAEFHMWNYHSHVFSVGDTFSLAMHLQYKIHEAPFDLLLEWLYVPIDPTCQPMRLYSTCLYHPNAPQCLSHMNSGCTFTSPHLAQRVASTVYQNCEHADNYTAYCLGISHMEPSFGLILHDGGTTLKFVDTPESLSGLYVFVVYFNGHVEAVAYTVVSTVDHFVNAIEERGFPPTAGQPPATTKPKEITPVNPGTSPLLRYAAWTGGLAAVVLLCLVIFLICTAKRMRVKAYRVDKSPYNQSMYYAGLPVDDFEDSESTDTEEEFGNAIGGSHGGSSYTVYIDKTRALVPRGSSAHHHHHHHHHH